European Patent Specification EP 3 717 916 B1, published January 1, 2025. Title: Target interference suppressed anti-drug antibody assay. Applicant: F. Hoffmann-La Roche AG. The sequence listing filed with the application follows.

SEQUENCE LISTING (116 sequences)

SEQ ID NO: 1 - protein, 121 aa, Artificial Sequence
  CFA0305 VH
QSLEESGGDLVKPGASLAVTCTASGFSSSSSYYMCWVRQAPGKGLEWIGCIYTGSGATYYASWAKGRFTISKTSSTTVTLQMTSLTVADTATYFCASDGGYVTPTHAMYLWGPGTLVTVSS

SEQ ID NO: 2 - protein, 117 aa, Artificial Sequence
  CFA0307 VH
QSLEESGGGLVKPGASLTLTCKASGIDFSNFYYICWVRQAPGKGLDLIACIYTVSGYTYYASWAKGRLTISKTSSTTVTLQMTSLTAADTATYFCARDLHAGITNLWGPGTLVTVSS

SEQ ID NO: 3 - protein, 122 aa, Artificial Sequence
  CFA0366 VH
QSLEESGGDLVKPGASLSLTCTAAGLDFSSSYYMCWVRQAPGKGLEWIACIYAGSSGIIYYANWAKGRFTISRPSSTTVTLQMTSLTAADTATYFCATYPTYGDGGHAFNLWGPGTLVTVSS

SEQ ID NO: 4 - protein, 117 aa, Artificial Sequence
  CFA0501 VH
QSVEESGGRLVTPGTPLTLTCTASGFSLSSYYMNWVRQAPGKGLEWIGMIYGSGATYYASWAKGRFTISKTSSTTVDLKMTSLTTEDTATYFCARQIYSGDNNDNFWGPGTLVTVSS

SEQ ID NO: 5 - protein, 117 aa, Artificial Sequence; identical to SEQ ID NO: 4
  CFA0538 VH

SEQ ID NO: 6 - protein, 117 aa, Artificial Sequence
  CFA0599 VH
QSVEESGGRLVTPGTPLTLTCTVSGLSLSDNTMTWVRQAPGKGLEWIGIISFGGDAYYASWAKGRFPISKTSTTVDLRITSPTTEDTATYFCARVGAGNIFWYFDLWGPGTLVTVSS

SEQ ID NO: 7 - protein, 116 aa, Artificial Sequence
  CFA0666 VH
QSVEESGGRLVTPGTPLTLTCTVSGFSLSTYAMGWVRQAPGKGLEWIGTIDTGDNSFYANWAKGRFTISKTSTTVDLKITSPTAEDTATYFCARNDGSVYNLFNLWGPGTLVTVSS

SEQ ID NO: 8 - protein, 110 aa, Artificial Sequence
  CFA0672 VH
QSVEESGGRLVTPGTPLTLTCTASGFSLSGNAINWVRQAPGKGLEWIGCIYTGSDTTYYATWAKGRFTISKTSTTVDLKIASPTTEDTATYFCARGSGLWGPGTLVTVSS

SEQ ID NO: 9 - protein, 116 aa, Artificial Sequence
  CFA0675 VH
QSVEESGGRLVTPGTPLTLTCTVSGFSLSTYAMGWVRQAPGKGLEWIGTIDTGDNSFYANWAKGRFTISRTSTTVDLKITSPTAEDTATYFCARNDGSVYNLFNLWGPGTLVTVSS

SEQ ID NO: 10 - protein, 123 aa, Artificial Sequence
  305LO5 VH
QVQLVESGGGLVQPGGSLRLSCAASGFTSHSSYYVAWVRQAPGKGLEWVGAIYTGSGATYKASWAKGRFTISKDTSKNQVVLTMTNMDPVDTATYYCASDGGYDYPTHAMHYWGQGTLVTVSS

SEQ ID NO: 11 - protein, 110 aa, Artificial Sequence
  CFA0305 VL
DVVMTQTPASVSAAVGGTVTIKCQASQNIGSDLAWYQQKPGQPPRLLIYGASKLASGVSSRFSGSGSGKEFTLTISDLECADAVTYYCQCTFVGSSYGNAFGGGTEVVVK

SEQ ID NO: 12 - protein, 110 aa, Artificial Sequence
  CFA0307 VL
AIEMTQTPFSVSAAVGGTVTIKCQASQNIYSNLAWYQQKPGQRPKLLIYGASNLESGVPSRFKGSGSGTEYTLTISDLECADAATYYCLQGYSYSNVDDAFGGGTEVVVK

SEQ ID NO: 13 - protein, 112 aa, Artificial Sequence
  CFA0366 VL
AQVLTQTPSSVSAAVGGTVTINCQSSQSVYSSDYLSWYQQKPGQPPKLLIYEASKLASGVPPRFSGSGSGTQFTLTISGVQCDDAATYYCQGTYYSSGWYFAFGGGTEVVVK

SEQ ID NO: 14 - protein, 110 aa, Artificial Sequence
  CFA0501 VL
AYDMTQTPASVEVAVGGTVTINCQASESISNWLAWYQQKPGQRPKLLIYRASTLASGVSSRFKGSGSGTQFTLTISGVECDDAATYYCQQDYSSSNVDNTFGGGTKVVVE

SEQ ID NO: 15 - protein, 110 aa, Artificial Sequence
  CFA0538 VL
AYDMTQTPASVEVAVGGTVTINCQASESISNWLAWYQQKPGQRPKLLIYRASTLASGVSSRFKGSGSGTQFTLTISGVECDDAATYYCQQDYSSSNVDNTFGGGTTVVVE

SEQ ID NO: 16 - protein, 110 aa, Artificial Sequence
  CFA0599 VL
AYDMTQTPASVEVSVGGTVTIKCQASESIYSALAWYQQKPGQPPKLLIYSASTLASGVPSRFKGSGSGTEYTLTISDLECADAATYYCQQYYSSTNVHNSFGGGTTVVVE

SEQ ID NO: 17 - protein, 110 aa, Artificial Sequence
  CFA0666 VL
DVVMTQTPASVSAAVGGTVTIKCQASENIYSALSWYQQKPGLRPRLLIYYASTLASGVPSRFKGSRSGTEFTLTISDLECADAATYYCQQYYDINSVDNTFGGGTKVVVE

SEQ ID NO: 18 - protein, 111 aa, Artificial Sequence
  CFA0672 VL
DVVMTQTPASVSAPVGGTVTIKCQASQNIYSLLAWYQQKPGQPPKLLIYHTSDLASGVPSRFRGSGSGTEFTLTISDLECADAATYYCQCTAYGSSDVGGTFGGGTTVVVE

SEQ ID NO: 19 - protein, 110 aa, Artificial Sequence
  CFA0675 VL
DVVMTQTPASVSAAVGGTVTIKCQASENIYSALSWYQQKPGLRPRLLIYYASTLASGVPSRFKGSRSGTEFTLTISDLECADAASYYCQQYYDINSVDNTFGGGTKVVVE

SEQ ID NO: 20 - protein, 110 aa, Artificial Sequence
  305LO5 VL
DVVMTQSPSSLSASVGDRVTITCQASQNIGSSLAWYQQKPGQAPRLLIYGASKTHSGVPSRFSGSGSGTDFTLTISSLQPEDVATYYCQSTKVGSSYGNHFGGGTKVEIK

SEQ ID NO: 21 - protein, 117 aa, Artificial Sequence
  CFA0330 VH
QSLEESGGDLVEPGASLTLTCTASGFSWNSGYDMCWVRQAPGKGLEWIACIYTGSSANTAYANWAKGRFTISKTSSTTVTLQMTGLTAADTATYFCARHDDYFFDLWGPGTLVTVSS

SEQ ID NO: 22 - protein, 115 aa, Artificial Sequence
  CFA0341 VH
QSVEESGGRLVTPGTPLTLTCTVSGIDLSSYTMGWVRQAPGKGLECIGYIHSFGSTYYASWAKGRFTISKTSTTVDLEITSPTTEDTATYFCARDVGGSSGWDLWGQGTLVTVSS

SEQ ID NO: 23 - protein, 116 aa, Artificial Sequence
  CFA0329 VH
QSLEESGGGLVKPGASLTLTCTASGFSFSSGYYMCWVRQAPGKGLEWIGCIGTISDSTYYASWAKGRFPISKASSTTVTLQMTSLTAADTATYFCARDPYSYGDLWGPGTLVTVSS

SEQ ID NO: 24 - protein, 114 aa, Artificial Sequence
  CFA0330 VL
DVVMTQTPASVSESVGGTVTINCQASQSIGNNLAWYQQKPGQPPKLLIYDASNLASGVPSRFKGSRSGTEPTLTNTLTISGVQCADVATYYCQSGWYGNSYVAAFGGGTEVVVK

SEQ ID NO: 25 - protein, 112 aa, Artificial Sequence
  CFA0341 VL
DVVMTQTPSSVSAAVGGTVTIKCQASENIYSNLAWYQQKPGQPPKRLIYDASDLASGVPSRFSGSGYGTQFTLTISGVQCEDAATYYCQANYDSTSSSFGNVFGGGTEVVVK

SEQ ID NO: 26 - protein, 110 aa, Artificial Sequence
  CFA0329 VL
DLVMTQTPASVSEPVGGTVTIKCQASQSIGTYLAWYQQKPGQPPKLLIYRASTLASGVPSRFKGSGSGTQFTLTISDLECADAATYYCLGGYYGFSYGNAFGGGTEVVVK

SEQ ID NO: 27 - protein, 325 aa, Artificial Sequence
  F760G4
ASTKGPSVFPLAPCSRSTSESTAALGCLVKDYFPEPVTVSWNSGALTSGVHTFPAVLQSSGLYSLSSVVTVPSSSLGTKTYTCNVDHKPSNTKVDKRVESKYGPPCPPCPAPEFRGGPKVFLFPPKPKDTLMISRTPEVTCVVVDVSQEDPEVQFNWYVDGVEVHNAKTKPREEQFNSTYRVVSVLTVLHQDWLNGKEYKCKVSNKGLPSSIEKTISKAKGQPREPQVYTLPPSQEEMTKNQVSLTCLVKGFYPSDIAVEWESNGQPENNYKTTPPVLDSDGSFFLYSRLTVDKSRWQEGNVFSCSVMHEALHNHYTQKSLSLSL

SEQ ID NO: 28 - protein, 325 aa, Artificial Sequence
  F939G4
ASTKGPSVFPLAPCSRSTSESTAALGCLVKDYFPEPVTVSWNSGALTSGVHTFPAVLQSSGLYSLSSVVTVPSSSLGTKTYTCNVDHKPSNTKVDKRVESKYGPPCPPCPAPEFRGGPKVFLFPPKPKDTLYISRTPEVTCVVVDVSQEDPEVQFNWYVDGVEVHNAKTKPREEQFNSTYRVVSVLTVLHQDWLNGKEYKCKVSNKGLPSSIEKTISKAKGQPREPQVYTLPPSQEEMTKNQVSLTCLVKGFYPSDIAVEWESNGQPENNYKTTPPVLDSDGSFFLYSRLTVDKSRWQEGNVFSCSVMHEALHYHVTQKSLSLSL

SEQ ID NO: 29 - protein, 325 aa, Artificial Sequence
  SG402
ASTKGPSVFPLAPCSRSTSESTAALGCLVKDYFPEPVTVSWNSGALTSGVHTFPAVLQSSGLYSLSSVVTVPSSSLGTKTYTCNVDHKPSNTKVDKRVESKYGPPCPPCPAPEFRGGPKVFLFPPKPKDTLMISRTPEVTCVVVDVSQEDPEVQFNWYVDGVEVHNAKTKPREEQFNSTYRVVSVLTVLHQDWLNGKEYKCKVSNKGLPSSIEKTISKAKGQPREPQVYTLPPSQEEMTKNQVSLTCLVKGFYPSDIAVEWESNGQPENNYKTTPPVLDSDGSFFLYSKLTVDKSRWQEGNVFSCSVMHEALHNHYTQKSLSLSP

SEQ ID NO: 30 - protein, 1676 aa, Artificial Sequence
  human C5
MGLLGILCFLIFLGKTWGQEQTYVISAPKIFRVGASENIVIQVYGYTEAFDATISIKSYPDKKFSYSSGHVHLSSENKFQNSAILTIQPKQLPGGQNPVSYVYLEVVSKHFSKSKRMPITYDNGFLFIHTDKPVYTPDQSVKVRVYSLNDDLKPAKRETVLTFIDPEGSEVDMVEEIDHIGIISFPDFKIPSNPRYGMWTIKAKYKEDFSTTGTAYFEVKEYVLPHFSVSIEPEYNFIGYKNFKNFEITIKARYFYNKVVTEADVYITFGIREDLKDDQKEMMQTAMQNTMLINGIAQVTFDSETAVKELSYYSLEDLNNKYLYIAVTVIESTGGFSEEAEIPGIKYVLSPYKLNLVATPLFLKPGIPYPIKVQVKDSLDQLVGGVPVTLNAQTIDVNQETSDLDPSKSVTRVDDGVASFVLNLPSGVTVLEFNVKTDAPDLPEENQAREGYRAIAYSSLSQSYLYIDWTDNHKALLVGEHLNIIVTPKSPYIDKITHYNYLILSKGKIIHFGTREKFSDASYQSINIPVTQNMVPSSRLLVYYIVTGEQTAELVSDSVWLNIEEKCGNQLQVHLSPDADAYSPGQTVSLNMATGMDSWVALAAVDSAVYGVQRGAKKPLERVFQFLEKSDLGCGAGGGLNNANVFHLAGLTFLTNANADDSQENDEPCKEILRPRRTLQKKIEEIAAKYKHSVVKKCCYDGACVNNDETCEQRAARISLGPRCIKAFTECCVVASQLRANISHKDMQLGRLHMKTLLPVSKPEIRSYFPESWLWEVHLVPRRKQLQFALPDSLTTWEIQGVGISNTGICVADTVKAKVFKDVFLEMNIPYSVVRGEQIQLKGTVYNYRTSGMQFCVKMSAVEGICTSESPVIDHQGTKSSKCVRQKVEGSSSHLVTFTVLPLEIGLHNINFSLETWFGKEILVKTLRVVPEGVKRESYSGVTLDPRGIYGTISRRKEFPYRIPLDLVPKTEIKRILSVKGLLVGEILSAVLSQEGINILTHLPKGSAEAELMSVVPVFYVFHYLETGNHWNIFHSDPLIEKQKLKKKLKEGMLSIMSYRNADYSYSVWKGGSASTWLTAFALRVLGQVNKYVEQNQNSICNSLLWLVENYQLDNGSFKENSQYQPIKLQGTLPVEARENSLYLTAFTVIGIRKAFDICPLVKIDTALIKADNFLLENTLPAQSTFTLAISAYALSLGDKTHPQFRSIVSALKREALVKGNPPIYRFWKDNLQHKDSSVPNTGTARMVETTAYALLTSLNLKDINYVNPVIKWLSEEQRYGGGFYSTQDTINAIEGLTEYSLLVKQLRLSMDIDVSYKHKGALHNYKMTDKNFLGRPVEVLLNDDLIVSTGFGSGLATVHVTTVVHKTSTSEEVCSFYLKIDTQDIEASHYRGYGNSDYKRIVACASYKPSREESSSGSSHAVMDISLPTGISANEEDLKALVEGVDQLFTDYQIKDGHVILQLNSIPSSDFLCVRFRIFELFEVGFLSPATFTVYEYHRPDKQCTMFYSTSNIKIQKVCEGAACKCVEADCGQMQEELDLTISAETRKQTACKPEIAYAYKVSITSITVENVFVKYKATLLDIYKTGEAVAEKDSEITFIKKVTCTNAELVKGRQYLIMGKEALQIKYNFSFRYIYPLDSLTWIEYWPRDTTCSSCQAFLANLDEFAEDIFLNGC

SEQ ID NO: 31 - protein, 673 aa, Artificial Sequence
  human C5, beta chain
MGLLGILCFLIFLGKTWGQEQTYVISAPKIFRVGASENIVIQVYGYTEAFDATISIKSYPDKKFSYSSGHVHLSSENKFQNSAILTIQPKQLPGGQNPVSYVYLEVVSKHFSKSKRMPITYDNGFLFIHTDKPVYTPDQSVKVRVYSLNDDLKPAKRETVLTFIDPEGSEVDMVEEIDHIGIISFPDFKIPSNPRYGMWTIKAKYKEDFSTTGTAYFEVKEYVLPHFSVSIEPEYNFIGYKNFKNFEITIKARYFYNKVVTEADVYITFGIREDLKDDQKEMMQTAMQNTMLINGIAQVTFDSETAVKELSYYSLEDLNNKYLYIAVTVIESTGGFSEEAEIPGIKYVLSPYKLNLVATPLFLKPGIPYPIKVQVKDSLDQLVGGVPVTLNAQTIDVNQETSDLDPSKSVTRVDDGVASFVLNLPSGVTVLEFNVKTDAPDLPEENQAREGYRAIAYSSLSQSYLYIDWTDNHKALLVGEHLNIIVTPKSPYIDKITHYNYLILSKGKIIHFGTREKFSDASYQSINIPVTQNMVPSSRLLVYYIVTGEQTAELVSDSVWLNIEEKCGNQLQVHLSPDADAYSPGQTVSLNMATGMDSWVALAAVDSAVYGVQRGAKKPLERVFQFLEKSDLGCGAGGGLNNANVFHLAGLTFLTNANADDSQENDEPCKEIL

SEQ ID NO: 32 - protein, 105 aa, Artificial Sequence
  human C5, MG1
EQTYVISAPKIFRVGASENIVIQVYGYTEAFDATISIKSYPDKKFSYSSGHVHLSSENKFQNSAILTIQPKQLPGGQNPVSYVYLEVVSKHFSKSKRMPITYDNG

SEQ ID NO: 33 - protein, 101 aa, Artificial Sequence
  human C5, MG2
FLFIHTDKPVYTPDQSVKVRVYSLNDDLKPAKRETVLTFIDPEGSEVDMVEEIDHIGIISFPDFKIPSNPRYGMWTIKAKYKEDFSTTGTAYFEVKEYVLP

SEQ ID NO: 34 - protein, 225 aa, Artificial Sequence
  human C5, MG1-MG2
MGLLGILCFLIFLGKTWGQEQTYVISAPKIFRVGASENIVIQVYGYTEAFDATISIKSYPDKKFSYSSGHVHLSSENKFQNSAILTIQPKQLPGGQNPVSYVYLEVVSKHFSKSKRMPITYDNGFLFIHTDKPVYTPDQSVKVRVYSLNDDLKPAKRETVLTFIDPEGSEVDMVEEIDHIGIISFPDFKIPSNPRYGMWTIKAKYKEDFSTTGTAYFEVKEYVLP

SEQ ID NO: 35 - protein, 1676 aa, Artificial Sequence
  cynomolgus C5
MGLLGILCFLIFLGKTWGQEQTYVISAPKIFRVGASENIVIQVYGYTEAFDATISIKSYPDKKFSYSSGHVHLSSENKFQNSAVLTIQPKQLPGGQNQVSYVYLEVVSKHFSKSKKIPITYDNGFLFIHTDKPVYTPDQSVKVRVYSLNDDLKPAKRETVLTFIDPEGSEIDMVEEIDHIGIISFPDFKIPSNPRYGMWTIQAKYKEDFSTTGTAFFEVKEYVLPHFSVSVEPESNFIGYKNFKNFEITIKARYFYNKVVTEADVYITFGIREDLKDDQKEMMQTAMQNTMLINGIAEVTFDSETAVKELSYYSLEDLNNKYLYIAVTVIESTGGFSEEAEIPGIKYVLSPYKLNLVATPLFLKPGIPYSIKVQVKDALDQLVGGVPVTLNAQTIDVNQETSDLEPRKSVTRVDDGVASFVVNLPSGVTVLEFNVKTDAPDLPDENQAREGYRAIAYSSLSQSYLYIDWTDNHKALLVGEYLNIIVTPKSPYIDKITHYNYLILSKGKIIHFGTREKLSDASYQSINIPVTQNMVPSSRLLVYYIVTGEQTAELVSDSVWLNIEEKCGNQLQVHLSPDADTYSPGQTVSLNMVTGMDSWVALTAVDSAVYGVQRRAKKPLERVFQFLEKSDLGCGAGGGLNNANVFHLAGLTFLTNANADDSQENDEPCKEIIRPRRMLQEKIEEIAAKYKHLVVKKCCYDGVRINHDETCEQRAARISVGPRCVKAFTECCVVASQLRANNSHKDLQLGRLHMKTLLPVSKPEIRSYFPESWLWEVHLVPRRKQLQFALPDSVTTWEIQGVGISNSGICVADTIKAKVFKDVFLEMNIPYSVVRGEQVQLKGTVYNYRTSGMQFCVKMSAVEGICTSESPVIDHQGTKSSKCVRQKVEGSSNHLVTFTVLPLEIGLQNINFSLETSFGKEILVKSLRVVPEGVKRESYSGITLDPRGIYGTISRRKEFPYRIPLDLVPKTEIKRILSVKGLLVGEILSAVLSREGINILTHLPKGSAEAELMSVVPVFYVFHYLETGNHWNIFHSDPLIEKRNLEKKLKEGMVSIMSYRNADYSYSVWKGGSASTWLTAFALRVLGQVHKYVEQNQNSICNSLLWLVENYQLDNGSFKENSQYQPIKLQGTLPVEARENSLYLTAFTVIGIRKAFDICPLVKINTALIKADTFLLENTLPAQSTFTLAISAYALSLGDKTHPQFRSIVSALKREALVKGNPPIYRFWKDSLQHKDSSVPNTGTARMVETTAYALLTSLNLKDINYVNPIIKWLSEEQRYGGGFYSTQDTINAIEGLTEYSLLVKQLRLNMDIDVAYKHKGPLHNYKMTDKNFLGRPVEVLLNDDLVVSTGFGSGLATVHVTTVVHKTSTSEEVCSFYLKIDTQDIEASHYRGYGNSDYKRIVACASYKPSKEESSSGSSHAVMDISLPTGINANEEDLKALVEGVDQLFTDYQIKDGHVILQLNSIPSSDFLCVRFRIFELFEVGFLSPATFTVYEYHRPDKQCTMFYSTSNIKIQKVCEGATCKCIEADCGQMQKELDLTISAETRKQTACNPEIAYAYKVIITSITTENVFVKYKATLLDIYKTGEAVAEKDSEITFIKKVTCTNAELVKGRQYLIMGKEALQIKYNFTFRYIYPLDSLTWIEYWPRDTTCSSCQAFLANLDEFAEDIFLNGC

SEQ ID NO: 36 - protein, 6 aa, Artificial Sequence
  CFA0305 HVR-H1
SSYYMC

SEQ ID NO: 37 - protein, 6 aa, Artificial Sequence
  CFA0307 HVR-H1
NFYYIC

SEQ ID NO: 38 - protein, 6 aa, Artificial Sequence
  CFA0366 HVR-H1
SSYYMC

SEQ ID NO: 39 - protein, 6 aa, Artificial Sequence
  CFA0501 HVR-H1
SSYYMN

SEQ ID NO: 40 - protein, 6 aa, Artificial Sequence
  CFA0538 HVR-H1
SSYYMN

SEQ ID NO: 41 - protein, 5 aa, Artificial Sequence
  CFA0599 HVR-H1
DNTMT

SEQ ID NO: 42 - protein, 5 aa, Artificial Sequence
  CFA0666 HVR-H1
TYAMG

SEQ ID NO: 43 - protein, 5 aa, Artificial Sequence
  CFA0672 HVR-H1
GNAIN

SEQ ID NO: 44 - protein, 5 aa, Artificial Sequence
  CFA0675 HVR-H1
TYAMG

SEQ ID NO: 45 - protein, 6 aa, Artificial Sequence
  305LO5 HVR-H1
SSYYVA

SEQ ID NO: 46 - protein, 17 aa, Artificial Sequence
  CFA0305 HVR-H2
CIYTGSGATYYASWAKG

SEQ ID NO: 47 - protein, 17 aa, Artificial Sequence
  CFA0307 HVR-H2
CIYTVSGYTYYASWAKG

SEQ ID NO: 48 - protein, 18 aa, Artificial Sequence
  CFA0366 HVR-H2
CIYAGSSGIIYYANWAKG

SEQ ID NO: 49 - protein, 16 aa, Artificial Sequence
  CFA0501 HVR-H2
MIYGSGATYYASWAKG

SEQ ID NO: 50 - protein, 16 aa, Artificial Sequence
  CFA0538 HVR-H2
MIYGSGATYYASWAKG

SEQ ID NO: 51 - protein, 16 aa, Artificial Sequence
  CFA0599 HVR-H2
IISFGGDAYYASWAKG

SEQ ID NO: 52 - protein, 16 aa, Artificial Sequence
  CFA0666 HVR-H2
TIDTGDNSFYANWAKG

SEQ ID NO: 53 - protein, 17 aa, Artificial Sequence
  CFA0672 HVR-H2
CIYTGSDTTYYATWAKG

SEQ ID NO: 54 - protein, 16 aa, Artificial Sequence
  CFA0675 HVR-H2
TIDTGDNSFYANWAKG

SEQ ID NO: 55 - protein, 17 aa, Artificial Sequence
  305LO5 HVR-H2
AIYTGSGATYKASWAKG

SEQ ID NO: 56 - protein, 13 aa, Artificial Sequence
  CFA0305 HVR-H3
DGGYVTPTHAMYL

SEQ ID NO: 57 - protein, 9 aa, Artificial Sequence
  CFA0307 HVR-H3
DLHAGITNL

SEQ ID NO: 58 - protein, 13 aa, Artificial Sequence
  CFA0366 HVR-H3
YPTYGDGGHAFNL

SEQ ID NO: 59 - protein, 11 aa, Artificial Sequence
  CFA0501 HVR-H3
QIYSGDNNDNF

SEQ ID NO: 60 - protein, 11 aa, Artificial Sequence
  CFA0538 HVR-H3
QIYSGDNNDNF

SEQ ID NO: 61 - protein, 12 aa, Artificial Sequence
  CFA0599 HVR-H3
VGAGNIFWYFDL

SEQ ID NO: 62 - protein, 11 aa, Artificial Sequence
  CFA0666 HVR-H3
NDGSVYNLFNL

SEQ ID NO: 63 - protein, 4 aa, Artificial Sequence
  CFA0672 HVR-H3
GSGL

SEQ ID NO: 64 - protein, 11 aa, Artificial Sequence
  CFA0675 HVR-H3
NDGSVYNLFNL

SEQ ID NO: 65 - protein, 13 aa, Artificial Sequence
  305LO5 HVR-H3
DGGYDYPTHAMHY

SEQ ID NO: 66 - protein, 11 aa, Artificial Sequence
  CFA0305 HVR-L1
QASQNIGSDLA

SEQ ID NO: 67 - protein, 11 aa, Artificial Sequence
  CFA0307 HVR-L1
QASQNIYSNLA

SEQ ID NO: 68 - protein, 13 aa, Artificial Sequence
  CFA0366 HVR-L1
QSSQSVYSSDYLS

SEQ ID NO: 69 - protein, 11 aa, Artificial Sequence
  CFA0501 HVR-L1
QASESISNWLA

SEQ ID NO: 70 - protein, 11 aa, Artificial Sequence
  CFA0538 HVR-L1
QASESISNWLA

SEQ ID NO: 71 - protein, 11 aa, Artificial Sequence
  CFA0599 HVR-L1
QASESIYSALA

SEQ ID NO: 72 - protein, 11 aa, Artificial Sequence
  CFA0666 HVR-L1
QASENIYSALS

SEQ ID NO: 73 - protein, 11 aa, Artificial Sequence
  CFA0672 HVR-L1
QASQNIYSLLA

SEQ ID NO: 74 - protein, 11 aa, Artificial Sequence
  CFA0675 HVR-L1
QASENIYSALS

SEQ ID NO: 75 - protein, 11 aa, Artificial Sequence
  305LO5 HVR-L1
QASQNIGSSLA

SEQ ID NO: 76 - protein, 7 aa, Artificial Sequence
  CFA0305 HVR-L2
GASKLAS

SEQ ID NO: 77 - protein, 7 aa, Artificial Sequence
  CFA0307 HVR-L2
GASNLES

SEQ ID NO: 78 - protein, 7 aa, Artificial Sequence
  CFA0366 HVR-L2
EASKLAS

SEQ ID NO: 79 - protein, 7 aa, Artificial Sequence
  CFA0501 HVR-L2
RASTLAS

SEQ ID NO: 80 - protein, 7 aa, Artificial Sequence
  CFA0538 HVR-L2
RASTLAS

SEQ ID NO: 81 - protein, 7 aa, Artificial Sequence
  CFA0599 HVR-L2
SASTLAS

SEQ ID NO: 82 - protein, 7 aa, Artificial Sequence
  CFA0666 HVR-L2
YASTLAS

SEQ ID NO: 83 - protein, 7 aa, Artificial Sequence
  CFA0672 HVR-L2
HTSDLAS

SEQ ID NO: 84 - protein, 7 aa, Artificial Sequence
  CFA0675 HVR-L2
YASTLAS

SEQ ID NO: 85 - protein, 7 aa, Artificial Sequence
  305LO5 HVR-L2
GASKTHS

SEQ ID NO: 86 - protein, 12 aa, Artificial Sequence
  CFA0305 HVR-L3
QCTFVGSSYGNA

SEQ ID NO: 87 - protein, 12 aa, Artificial Sequence
  CFA0307 HVR-L3
LQGYSYSNVDDA

SEQ ID NO: 88 - protein, 12 aa, Artificial Sequence
  CFA0366 HVR-L3
QGTYYSSGWYFA

SEQ ID NO: 89 - protein, 12 aa, Artificial Sequence
  CFA0501 HVR-L3
QQDYSSSNVDNT

SEQ ID NO: 90 - protein, 12 aa, Artificial Sequence
  CFA0538 HVR-L3
QQDYSSSNVDNT

SEQ ID NO: 91 - protein, 12 aa, Artificial Sequence
  CFA0599 HVR-L3
QQYYSSTNVHNS

SEQ ID NO: 92 - protein, 12 aa, Artificial Sequence
  CFA0666 HVR-L3
QQYYDINSVDNT

SEQ ID NO: 93 - protein, 13 aa, Artificial Sequence
  CFA0672 HVR-L3
QCTAYGSSDVGGT

SEQ ID NO: 94 - protein, 12 aa, Artificial Sequence
  CFA0675 HVR-L3
QQYYDINSVDNT

SEQ ID NO: 95 - protein, 12 aa, Artificial Sequence
  305LO5 HVR-L3
QSTKVGSSYGNH

SEQ ID NO: 96 - protein, 1680 aa, Artificial Sequence
  mouse C5
MGLWGILCLLIFLDKTWGQEQTYVISAPKILRVGSSENVVIQVHGYTEAFDATLSLKSYPDKKVTFSSGYVNLSPENKFQNAALLTLQPNQVPREESPVSHVYLEVVSKHFSKSKKIPITYNNGILFIHTDKPVYTPDQSVKIRVYSLGDDLKPAKRETVLTFIDPEGSEVDIVEENDYTGIISFPDFKIPSNPKYGVWTIKANYKKDFTTTGTAYFEIKEYVLPRFSVSIELERTFIGYKNFKNFEITVKARYFYNKVVPDAEVYAFFGLREDIKDEEKQMMHKATQAAKLVDGVAQISFDSETAVKELSYNSLEDLNNKYLYIAVTVTESSGGFSEEAEIPGVKYVLSPYTLNLVATPLFVKPGIPFSIKAQVKDSLEQAVGGVPVTLMAQTVDVNQETSDLETKRSITHDTDGVAVFVLNLPSNVTVLKFEIRTDDPELPEENQASKEYEAVAYSSLSQSYIYIAWTENYKPMLVGEYLNIMVTPKSPYIDKITHYNYLILSKGKIVQYGTREKLFSSTYQNINIPVTQNMVPSARLLVYYIVTGEQTAELVADAVWINIEEKCGNQLQVHLSPDEYVYSPGQTVSLDMVTEADSWVALSAVDRAVYKVQGNAKRAMQRVFQALDEKSDLGCGAGGGHDNADVFHLAGLTFLTNANADDSHYRDDSCKEILRSKRNLHLLRQKIEEQAAKYKHSVPKKCCYDGARVNFYETCEERVARVTIGPLCIRAFNECCTIANKIRKESPHKPVQLGRIHIKTLLPVMKADIRSYFPESWLWEIHRVPKRKQLQVTLPDSLTTWEIQGIGISDNGICVADTLKAKVFKEVFLEMNIPYSVVRGEQIQLKGTVYNYMTSGTKFCVKMSAVEGICTSGSSAASLHTSRPSRCVFQRIEGSSSHLVTFTLLPLEIGLHSINFSLETSFGKDILVKTLRVVPEGVKRESYAGVILDPKGIRGIVNRRKEFPYRIPLDLVPKTKVERILSVKGLLVGEFLSTVLSKEGINILTHLPKGSAEAELMSIAPVFYVFHYLEAGNHWNIFYPDTLSKRQSLEKKIKQGVVSVMSYRNADYSYSMWKGASASTWLTAFALRVLGQVAKYVKQDENSICNSLLWLVEKCQLENGSFKENSQYLPIKLQGTLPAEAQEKTLYLTAFSVIGIRKAVDICPTMKIHTALDKADSFLLENTLPSKSTFTLAIVAYALSLGDRTHPRFRLIVSALRKEAFVKGDPPIYRYWRDTLKRPDSSVPSSGTAGMVETTAYALLASLKLKDMNYANPIIKWLSEEQRYGGGFYSTQDTINAIEGLTEYSLLLKQIHLDMDINVAYKHEGDFHKYKVTEKHFLGRPVEVSLNDDLVVSTGYSSGLATVYVKTVVHKISVSEEFCSFYLKIDTQDIEASSHFRLSDSGFKRIIACASYKPSKEESTSGSSHAVMDISLPTGIGANEEDLRALVEGVDQLLTDYQIKDGHVILQLNSIPSRDFLCVRFRIFELFQVGFLNPATFTVYEYHRPDKQCTMIYSISDTRLQKVCEGAACTCVEADCAQLQAEVDLAISADSRKEKACKPETAYAYKVRITSATEENVFVKYTATLLVTYKTGEAADENSEVTFIKKMSCTNANLVKGKQYLIMGKEVLQIKHNFSFKYIYPLDSSTWIEYWPTDTTCPSCQAFVENLNNFAEDLFLNSCE

SEQ ID NO: 97 - protein, 123 aa, Artificial Sequence [sequence omitted]

SEQ ID NO: 98 - protein, 123 aa, Artificial Sequence
  305LO16 VH
QVQLVESGGGLVQPGRSLRLSCAASGFTVHSSYYMAWVRQAPGKGLEWVGAIFTGSGAEYKAEWVKGRFTISRDNSKNTLYLQMNSLRAEDTAVYYCASDAGYDYPTHAMHYWGRGTLVTVSS

SEQ ID NO: 99 - protein, 123 aa, Artificial Sequence
  305LO18 VH
QVQLVESGGGLVQPGRSLRLSCAASGFTVHSSYYMAWVRQAPGKGLEWVGAIFTGSGAEYKAEWAKGRVTISKDTSKNQVVLTMTNMDPVDTATYYCASDAGYDYPTHAMHYWGRGTLVTVSS

SEQ ID NO: 100 - protein, 123 aa, Artificial Sequence
  305LO19, 20, 22 VH
QVQLVESGGGLVQPGGSLRLSCAASGFTVHSSYYMAWVRQAPGKGLEWVGAIFTGSGAEYKAEWAKGRVTISKDTSKNQVVLTMTNMDPVDTATYYCASDAGYDYPTHAMHYWGQGTLVTVSS

SEQ ID NO: 101 - protein, 123 aa, Artificial Sequence
  305LO23 VH
QVQLVESGGGLVQPGGSLRLSCAASGFTVHSSYYMAWVRQAPGKGLEWVSGIFTGSGATYKAEWAKGRVTISKDTSKNQVVLTMTNMDPVDTATYYCASDAGYDYPTHAMHYWGQGTLVTVSS

SEQ ID NO: 102 - protein, 110 aa, Artificial Sequence [sequence omitted]

SEQ ID NO: 103 - protein, 110 aa, Artificial Sequence
  305LO20 VL
DIQMTQSPSSLSASVGDRVTITCRASQGISSSLAWYQQKPGQAPRLLIYGASETESGVPSRFSGSGSGTDFTLTISSLQPEDFATYYCQNTKVGSSYGNTFGGGTKVEIK

SEQ ID NO: 104 - protein, 110 aa, Artificial Sequence
  305LO22, 23 VL
DIQMTQSPSSLSASVGDRVTITCRASQGISSSLAWYQQKPGQAPRLLIYGASTTQSGVPSRFSGSGSGTDFTLTISSLQPEDFATYYCQNTKVGSSYGNTFGGGTKVEIK

SEQ ID NO: 105 - protein, 328 aa, Artificial Sequence
  SG115
ASTKGPSVFPLAPSSKSTSGGTAALGCLVKDYFPEPVTVSWNSGALTSGVHTFPAVLQSSGLYSLSSVVTVPSSSLGTQTYICNVNHKPSNTKVDKKVEPKSCDKTHTCPPCPAPELRRGPKVFLFPPKPKDTLMISRTPEVTCVVVDVSHEDPEVKFNWYVDGVEVHNAKTKPREEQYNSTYRVVSVLTVLHQDWLNGKEYKCKVSNKGLPSSIEKTISKAKGQPREPQVYTLPPSREEMTKNQVSLTCLVKGFYPSDIAVEWESNGQPENNYKTTPPVLDSDGSFFLYSKLTVDKSRWQQGNVFSCSVLHEALHAHYTRKELSLSP

SEQ ID NO: 106 - protein, 325 aa, Artificial Sequence
  SG422
ASTKGPSVFPLAPCSRSTSGGTAALGCLVKDYFPEPVTVSWNSGALTSGVHTFPAVLQSSGLYSLSSVVTVPSSSLGTKTYTCNVDHKPSNTKVDKRVESKYGPPCPPCPAPEFRRGPKVFLFPPKPKDTLMISRTPEVTCVVVDVSHEDPEVKFNWYVDGVEVHNAKTKPREEQYNSTYRVVSVLTVLHQDWLNGKEYKCKVSNKGLPSSIEKTISKAKGQPREPQVYTLPPSREEMTKNQVSLTCLVKGFYPSDIAVEWESNGQPENNYKTTPPVLDSDGSFFLYSKLTVDKSRWQQGNVFSCSVLHEALHAHYTRKELSLSP

SEQ ID NO: 107 - protein, 325 aa, Artificial Sequence
  SG429
ASTKGPSVFPLAPCSRSTSGGTAALGCLVKDYFPEPVTVSWNSGALTSGVHTFPAVLQSSGLYSLSSVVTVPSSSLGTKTYTCNVDHKPSNTKVDKRVESKYGPPCPPCPAPEFRRGPKVFLFPPKPKDTLMISRTPEVTCVVVDVSHEDPEVKFNWYVDGVEVHNAKTKPREEQYNSTYRVVSVLTVLHQDWLNGKEYKCKVSNKGLPSSIEKTISKAKGQPREPQVYTLPPSREEMTKNQVSLTCLVKGFYPSDIAVEWESNGQPENNYKTTPPVLDSDGSFFLYSRLTVDKSRWQQGNVFSCSVLHEALHAHYTRKELSLSP

SEQ ID NO: 108 - protein, 6 aa, Artificial Sequence
  305LO15, 16, 18, 19, 20, 22, 23 HVR-H1
SSYYMA

SEQ ID NO: 109 - protein, 17 aa, Artificial Sequence
  305LO15, 18, 19, 20, 22 HVR-H2
AIFTGSGAEYKAEWAKG

SEQ ID NO: 110 - protein, 17 aa, Artificial Sequence
  305LO16 HVR-H2
AIFTGSGAEYKAEWVKG

SEQ ID NO: 111 - protein, 17 aa, Artificial Sequence
  305LO23 HVR-H2
GIFTGSGATYKAEWAKG

SEQ ID NO: 112 - protein, 13 aa, Artificial Sequence
  305LO15, 16, 18, 19, 20, 22, 23 HVR-H3
DAGYDYPTHAMHY

SEQ ID NO: 113 - protein, 11 aa, Artificial Sequence
  305LO15, 16, 18, 19, 20, 22, 23 HVR-L1
RASQGISSSLA

SEQ ID NO: 114 - protein, 7 aa, Artificial Sequence
  305LO15, 16, 18, 19, 20 HVR-L2
GASETES

SEQ ID NO: 115 - protein, 7 aa, Artificial Sequence
  305LO22, 23 HVR-L2
GASTTQS

SEQ ID NO: 116 - protein, 12 aa, Artificial Sequence
  305LO15, 16, 18, 19, 20, 22, 23 HVR-L3
QNTKVGSSYGNT